European Patent Application EP 4 660 206 A1, published December 10, 2025. Title: TCR MOLECULE TARGETING KRAS G12V MUTATION, AND CELL AND USE THEREOF. Applicant: BEIJING DCTY BIOTECH CO., LTD. The sequence listing filed with the application follows.

SEQUENCE LISTING (94 sequences)

SEQ ID NO: 1 - protein, 272 aa, synthetic construct
MRQVARVIVFLTLSTLSLAKTTQPISMDSYEGQEVNITCSHNNIATNDYITWYQQFPSQGPRFIIQGYKTKVTNEVASLFIPADRKSSTLSLPRVSLSDTAVYYCLVGALSSSWYGQNFVFGPGTRLSVLPYIQNPDPAVYQLRDSKSSDKSVCLFTDFDSQTNVSQSKDSDVYITDKTVLDMRSMDFKSNSAVAWSNKSDFACANAFNNSIIPEDTFFPSPESSCDVKLVEKSFETDTNLNFQNLSVIGFRILLLKVAGFNLLMTLRLWSS

SEQ ID NO: 2 - protein, 114 aa, synthetic construct
LAKTTQPISMDSYEGQEVNITCSHNNIATNDYITWYQQFPSQGPRFIIQGYKTKVTNEVASLFIPADRKSSTLSLPRVSLSDTAVYYCLVGALSSSWYGQNFVFGPGTRLSVLP

SEQ ID NO: 3 - protein, 7 aa, synthetic construct
NIATNDY

SEQ ID NO: 4 - protein, 5 aa, synthetic construct
GYKTK

SEQ ID NO: 5 - protein, 15 aa, synthetic construct
LVGALSSSWYGQNFV

SEQ ID NO: 6 - protein, 309 aa, synthetic construct
MGCRLLCCVVFCLLQAGPLDTAVSQTPKYLVTQMGNDKSIKCEQNLGHDTMYWYKQDSKKFLKIMFSYNNKELIINETVPNRFSPKSPDKAHLNLHINSLELGDSAVYFCASSQSGAQDGYTFGSGTRLTVVEDLNKVFPPEVAVFEPSEAEISHTQKATLVCLATGFFPDHVELSWWVNGKEVHSGVSTDPQPLKEQPALNDSRYCLSSRLRVSATFWQNPRNHFRCQVQFYGLSENDEWTQDRAKPVTQIVSAEAWGRADCGFTSVSYQQGVLSATILYEILLGKATLYAVLVSALVLMAMVKRKDF

SEQ ID NO: 7 - protein, 113 aa, synthetic construct
DTAVSQTPKYLVTQMGNDKSIKCEQNLGHDTMYWYKQDSKKFLKIMFSYNNKELIINETVPNRFSPKSPDKAHLNLHINSLELGDSAVYFCASSQSGAQDGYTFGSGTRLTVV

SEQ ID NO: 8 - protein, 5 aa, synthetic construct
LGHDT

SEQ ID NO: 9 - protein, 6 aa, synthetic construct
YNNKEL

SEQ ID NO: 10 - protein, 12 aa, synthetic construct
ASSQSGAQDGYT

SEQ ID NO: 11 - protein, 279 aa, synthetic construct
MAMLLGASVLILWLQPDWVNSQQKNDDQQVKQNSPSLSVQEGRISILNCDYTNSMFDYFLWYKKYPAEGPTFLISISSIKDKNEDGRFTVFLNKSAKHLSLHIVPSQPGDSAVYFCAAKDNAGNMLTFGGGTRLMVKPHIQNPDPAVYQLRDSKSSDKSVCLFTDFDSQTNVSQSKDSDVYITDKTVLDMRSMDFKSNSAVAWSNKSDFACANAFNNSIIPEDTFFPSPESSCDVKLVEKSFETDTNLNFQNLSVIGFRILLLKVAGFNLLMTLRLWSS

SEQ ID NO: 12 - protein, 112 aa, synthetic construct
DQQVKQNSPSLSVQEGRISILNCDYTNSMFDYFLWYKKYPAEGPTFLISISSIKDKNEDGRFTVFLNKSAKHLSLHIVPSQPGDSAVYFCAAKDNAGNMLTFGGGTRLMVKP

SEQ ID NO: 13 - protein, 6 aa, synthetic construct
NSMFDY

SEQ ID NO: 14 - protein, 7 aa, synthetic construct
ISSIKDK

SEQ ID NO: 15 - protein, 11 aa, synthetic construct
AAKDNAGNMLT

SEQ ID NO: 16 - protein, 307 aa, synthetic construct
MGSRLLCWVLLCLLGAGPVKAGVTQTPRYLIKTRGQQVTLSCSPISGHRSVSWYQQTPGQGLQFLFEYFSETQRNKGNFPGRFSGRQFSNSRSEMNVSTLELGDSALYLCASSLGTAEAFFGQGTRLTVVEDLNKVFPPEVAVFEPSEAEISHTQKATLVCLATGFFPDHVELSWWVNGKEVHSGVSTDPQPLKEQPALNDSRYCLSSRLRVSATFWQNPRNHFRCQVQFYGLSENDEWTQDRAKPVTQIVSAEAWGRADCGFTSVSYQQGVLSATILYEILLGKATLYAVLVSALVLMAMVKRKDF

SEQ ID NO: 17 - protein, 111 aa, synthetic construct
KAGVTQTPRYLIKTRGQQVTLSCSPISGHRSVSWYQQTPGQGLQFLFEYFSETQRNKGNFPGRFSGRQFSNSRSEMNVSTLELGDSALYLCASSLGTAEAFFGQGTRLTVV

SEQ ID NO: 18 - protein, 5 aa, synthetic construct
SGHRS

SEQ ID NO: 19 - protein, 6 aa, synthetic construct
YFSETQ

SEQ ID NO: 20 - protein, 10 aa, synthetic construct
ASSLGTAEAF

SEQ ID NO: 21 - protein, 277 aa, synthetic construct
MAMLLGASVLILWLQPDWVNSQQKNDDQQVKQNSPSLSVQEGRISILNCDYTNSMFDYFLWYKKYPAEGPTFLISISSIKDKNEDGRFTVFLNKSAKHLSLHIVPSQPGDSAVYFCAANSGYALNFGKGTSLLVTPHIQNPDPAVYQLRDSKSSDKSVCLFTDFDSQTNVSQSKDSDVYITDKTVLDMRSMDFKSNSAVAWSNKSDFACANAFNNSIIPEDTFFPSPESSCDVKLVEKSFETDTNLNFQNLSVIGFRILLLKVAGFNLLMTLRLWSS

SEQ ID NO: 22 - protein, 110 aa, synthetic construct
DQQVKQNSPSLSVQEGRISILNCDYTNSMFDYFLWYKKYPAEGPTFLISISSIKDKNEDGRFTVFLNKSAKHLSLHIVPSQPGDSAVYFCAANSGYALNFGKGTSLLVTP

SEQ ID NO: 23 - protein, 6 aa, synthetic construct
NSMFDY

SEQ ID NO: 24 - protein, 7 aa, synthetic construct
ISSIKDK

SEQ ID NO: 25 - protein, 9 aa, synthetic construct
AANSGYALN

SEQ ID NO: 26 - protein, 311 aa, synthetic construct
MGSRLLCWVLLCLLGAGPVKAGVTQTPRYLIKTRGQQVTLSCSPISGHRSVSWYQQTPGQGLQFLFEYFSETQRNKGNFPGRFSGRQFSNSRSEMNVSTLELGDSALYLCASSLGGVGNEQFFGPGTRLTVLEDLKNVFPPEVAVFEPSEAEISHTQKATLVCLATGFYPDHVELSWWVNGKEVHSGVSTDPQPLKEQPALNDSRYCLSSRLRVSATFWQNPRNHFRCQVQFYGLSENDEWTQDRAKPVTQIVSAEAWGRADCGFTSESYQQGVLSATILYEILLGKATLYAVLVSALVLMAMVKRKDSRG

SEQ ID NO: 27 - protein, 113 aa, synthetic construct
KAGVTQTPRYLIKTRGQQVTLSCSPISGHRSVSWYQQTPGQGLQFLFEYFSETQRNKGNFPGRFSGRQFSNSRSEMNVSTLELGDSALYLCASSLGGVGNEQFFGPGTRLTVL

SEQ ID NO: 28 - protein, 5 aa, synthetic construct
SGHRS

SEQ ID NO: 29 - protein, 6 aa, synthetic construct
YFSETQ

SEQ ID NO: 30 - protein, 12 aa, synthetic construct
ASSLGGVGNEQF

SEQ ID NO: 31 - protein, 275 aa, synthetic construct
MMKSLRVLLVILWLQLSWVWSQQKEVEQNSGPLSVPEGAIASLNCTYSDRGSQSFFWYRQYSGKSPELIMFIYSNGDKEDGRFTAQLNKASQYVSLLIRDSQPSDSATYLCAVERGSTLGRLYFGRGTQLTVWPDIQNPDPAVYQLRDSKSSDKSVCLFTDFDSQTNVSQSKDSDVYITDKTVLDMRSMDFKSNSAVAWSNKSDFACANAFNNSIIPEDTFFPSPESSCDVKLVEKSFETDTNLNFQNLSVIGFRILLLKVAGFNLLMTLRLWSS

SEQ ID NO: 32 - protein, 112 aa, synthetic construct
QKEVEQNSGPLSVPEGAIASLNCTYSDRGSQSFFWYRQYSGKSPELIMFIYSNGDKEDGRFTAQLNKASQYVSLLIRDSQPSDSATYLCAVERGSTLGRLYFGRGTQLTVWP

SEQ ID NO: 33 - protein, 6 aa, synthetic construct
DRGSQS

SEQ ID NO: 34 - protein, 6 aa, synthetic construct
IYSNGD

SEQ ID NO: 35 - protein, 12 aa, synthetic construct
AVERGSTLGRLY

SEQ ID NO: 36 - protein, 321 aa, synthetic construct
MGTSLLCWVVLGFLGTDSVSTDHTGAGVSQSPRYKVTKRGQDVTLRCDPISSHATLYWYQQALGQGPEFLTYFNYEAQPDKSGLPSDRFSAERPEGSISTLTIQRTEQRDSAMYRCASSLSSPTGGPINEQFFGPGTRLTVLEDLKNVFPPEVAVFEPSEAEISHTQKATLVCLATGFYPDHVELSWWVNGKEVHSGVSTDPQPLKEQPALNDSRYCLSSRLRVSATFWQNPRNHFRCQVQFYGLSENDEWTQDRAKPVTQIVSAEAWGRADCGFTSESYQQGVLSATILYEILLGKATLYAVLVSALVLMAMVKRKDSRG

SEQ ID NO: 37 - protein, 118 aa, synthetic construct
GAGVSQSPRYKVTKRGQDVTLRCDPISSHATLYWYQQALGQGPEFLTYFNYEAQPDKSGLPSDRFSAERPEGSISTLTIQRTEQRDSAMYRCASSLSSPTGGPINEQFFGPGTRLTVL

SEQ ID NO: 38 - protein, 5 aa, synthetic construct
SSHAT

SEQ ID NO: 39 - protein, 6 aa, synthetic construct
FNYEAQ

SEQ ID NO: 40 - protein, 16 aa, synthetic construct
ASSLSSPTGGPINEQF

SEQ ID NO: 41 - protein, 274 aa, synthetic construct
MKTFAGFSFLFLWLQLDCMSRGEDVEQSLFLSVREGDSSVINCTYTDSSSTYLYWYKQEPGAGLQLLTYIFSNMDMKQDQRLTVLLNKKDKHLSLRIADTQTGDSAIYFCAESPGGGADGLTFGKGTHLIIQPYIQNPDPAVYQLRDSKSSDKSVCLFTDFDSQTNVSQSKDSDVYITDKTVLDMRSMDFKSNSAVAWSNKSDFACANAFNNSIIPEDTFFPSPESSCDVKLVEKSFETDTNLNFQNLSVIGFRILLLKVAGFNLLMTLRLWSS

SEQ ID NO: 42 - protein, 112 aa, synthetic construct
GEDVEQSLFLSVREGDSSVINCTYTDSSSTYLYWYKQEPGAGLQLLTYIFSNMDMKQDQRLTVLLNKKDKHLSLRIADTQTGDSAIYFCAESPGGGADGLTFGKGTHLIIQP

SEQ ID NO: 43 - protein, 6 aa, synthetic construct
DSSSTY

SEQ ID NO: 44 - protein, 7 aa, synthetic construct
IFSNMDM

SEQ ID NO: 45 - protein, 12 aa, synthetic construct
AESPGGGADGLT

SEQ ID NO: 46 - protein, 309 aa, synthetic construct
MLLLLLLLGPGSGLGAVVSQHPSWVICKSGTSVKIECRSLDFQATTMFWYRQFPKQSLMLMATSNEGSKATYEQGVEKDKFLINHASLTLSTLTVTSAHPEDSSFYICSAPRGWAAGVYGYTFGSGTRLTVVEDLNKVFPPEVAVFEPSEAEISHTQKATLVCLATGFFPDHVELSWWVNGKEVHSGVSTDPQPLKEQPALNDSRYCLSSRLRVSATFWQNPRNHFRCQVQFYGLSENDEWTQDRAKPVTQIVSAEAWGRADCGFTSVSYQQGVLSATILYEILLGKATLYAVLVSALVLMAMVKRKDF

SEQ ID NO: 47 - protein, 118 aa, synthetic construct
GAVVSQHPSWVICKSGTSVKIECRSLDFQATTMFWYRQFPKQSLMLMATSNEGSKATYEQGVEKDKFLINHASLTLSTLTVTSAHPEDSSFYICSAPRGWAAGVYGYTFGSGTRLTVV

SEQ ID NO: 48 - protein, 6 aa, synthetic construct
DFQATT

SEQ ID NO: 49 - protein, 7 aa, synthetic construct
SNEGSKA

SEQ ID NO: 50 - protein, 14 aa, synthetic construct
SAPRGWAAGVYGYT

SEQ ID NO: 51 - protein, 275 aa, synthetic construct
MLLELIPLLGIHFVLRTARAQSVTQPDIHITVSEGASLELRCNYSYGATPYLFWYVQSPGQGLQLLLKYFSGDTLVQGIKGFEAEFKRSQSSFNLRKPSVHWSDAAEYFCAVGASREYGNKLVFGAGTILRVKSYIQNPDPAVYQLRDSKSSDKSVCLFTDFDSQTNVSQSKDSDVYITDKTVLDMRSMDFKSNSAVAWSNKSDFACANAFNNSIIPEDTFFPSPESSCDVKLVEKSFETDTNLNFQNLSVIGFRILLLKVAGFNLLMTLRLWSS

SEQ ID NO: 52 - protein, 115 aa, synthetic construct
AQSVTQPDIHITVSEGASLELRCNYSYGATPYLFWYVQSPGQGLQLLLKYFSGDTLVQGIKGFEAEFKRSQSSFNLRKPSVHWSDAAEYFCAVGASREYGNKLVFGAGTILRVKS

SEQ ID NO: 53 - protein, 6 aa, synthetic construct
YGATPY

SEQ ID NO: 54 - protein, 8 aa, synthetic construct
YFSGDTLV

SEQ ID NO: 55 - protein, 13 aa, synthetic construct
AVGASREYGNKLV

SEQ ID NO: 56 - protein, 307 aa, synthetic construct
MDTRVLCCAVICLLGAGLSNAGVMQNPRHLVRRRGQEARLRCSPMKGHSHVYWYRQLPEEGLKFMVYLQKENIIDESGMPKERFSAEFPKEGPSILRIQQVVRGDSAAYFCASSPGGLLHFGNGTRLTVTEDLNKVFPPEVAVFEPSEAEISHTQKATLVCLATGFFPDHVELSWWVNGKEVHSGVSTDPQPLKEQPALNDSRYCLSSRLRVSATFWQNPRNHFRCQVQFYGLSENDEWTQDRAKPVTQIVSAEAWGRADCGFTSVSYQQGVLSATILYEILLGKATLYAVLVSALVLMAMVKRKDF

SEQ ID NO: 57 - protein, 111 aa, synthetic construct
NAGVMQNPRHLVRRRGQEARLRCSPMKGHSHVYWYRQLPEEGLKFMVYLQKENIIDESGMPKERFSAEFPKEGPSILRIQQVVRGDSAAYFCASSPGGLLHFGNGTRLTVT

SEQ ID NO: 58 - protein, 5 aa, synthetic construct
KGHSH

SEQ ID NO: 59 - protein, 6 aa, synthetic construct
LQKENI

SEQ ID NO: 60 - protein, 9 aa, synthetic construct
ASSPGGLLH

SEQ ID NO: 61 - protein, 279 aa, synthetic construct
MAMLLGASVLILWLQPDWVNSQQKNDDQQVKQNSPSLSVQEGRISILNCDYTNSMFDYFLWYKKYPAEGPTFLISISSIKDKNEDGRFTVFLNKSAKHLSLHIVPSQPGDSAVYFCAGKTNTGNQFYFGTGTSLTVIPNIQNPDPAVYQLRDSKSSDKSVCLFTDFDSQTNVSQSKDSDVYITDKTVLDMRSMDFKSNSAVAWSNKSDFACANAFNNSIIPEDTFFPSPESSCDVKLVEKSFETDTNLNFQNLSVIGFRILLLKVAGFNLLMTLRLWSS

SEQ ID NO: 62 - protein, 112 aa, synthetic construct
DQQVKQNSPSLSVQEGRISILNCDYTNSMFDYFLWYKKYPAEGPTFLISISSIKDKNEDGRFTVFLNKSAKHLSLHIVPSQPGDSAVYFCAGKTNTGNQFYFGTGTSLTVIP

SEQ ID NO: 63 - protein, 6 aa, synthetic construct
NSMFDY

SEQ ID NO: 64 - protein, 7 aa, synthetic construct
ISSIKDK

SEQ ID NO: 65 - protein, 11 aa, synthetic construct
AGKTNTGNQFY

SEQ ID NO: 66 - protein, 307 aa, synthetic construct
MGSRLLCWVLLCLLGAGPVKAGVTQTPRYLIKTRGQQVTLSCSPISGHRSVSWYQQTPGQGLQFLFEYFSETQRNKGNFPGRFSGRQFSNSRSEMNVSTLELGDSALYLCASSSGHPEAFFGQGTRLTVVEDLNKVFPPEVAVFEPSEAEISHTQKATLVCLATGFFPDHVELSWWVNGKEVHSGVSTDPQPLKEQPALNDSRYCLSSRLRVSATFWQNPRNHFRCQVQFYGLSENDEWTQDRAKPVTQIVSAEAWGRADCGFTSVSYQQGVLSATILYEILLGKATLYAVLVSALVLMAMVKRKDF

SEQ ID NO: 67 - protein, 111 aa, synthetic construct
KAGVTQTPRYLIKTRGQQVTLSCSPISGHRSVSWYQQTPGQGLQFLFEYFSETQRNKGNFPGRFSGRQFSNSRSEMNVSTLELGDSALYLCASSSGHPEAFFGQGTRLTVV

SEQ ID NO: 68 - protein, 5 aa, synthetic construct
SGHRS

SEQ ID NO: 69 - protein, 6 aa, synthetic construct
YFSETQ

SEQ ID NO: 70 - protein, 10 aa, synthetic construct
ASSSGHPEAF

SEQ ID NO: 71 - protein, 273 aa, synthetic construct
METLLGVSLVILWLQLARVNSQQGEEDPQALSIQEGENATMNCSYKTSINNLQWYRQNSGRGLVHLILIRSNEREKHSGRLRVTLDTSKKSSSLLITASRAADTASYFCATDAGGGADGLTFGKGTHLIIQPYIQNPDPAVYQLRDSKSSDKSVCLFTDFDSQTNVSQSKDSDVYITDKTVLDMRSMDFKSNSAVAWSNKSDFACANAFNNSIIPEDTFFPSPESSCDVKLVEKSFETDTNLNFQNLSVIGFRILLLKVAGFNLLMTLRLWSS

SEQ ID NO: 72 - protein, 112 aa, synthetic construct
SQQGEEDPQALSIQEGENATMNCSYKTSINNLQWYRQNSGRGLVHLILIRSNEREKHSGRLRVTLDTSKKSSSLLITASRAADTASYFCATDAGGGADGLTFGKGTHLIIQP

SEQ ID NO: 73 - protein, 5 aa, synthetic construct
TSINN

SEQ ID NO: 74 - protein, 7 aa, synthetic construct
IRSNERE

SEQ ID NO: 75 - protein, 12 aa, synthetic construct
ATDAGGGADGLT

SEQ ID NO: 76 - protein, 310 aa, synthetic construct
MGFRLLCCVAFCLLGAGPVDSGVTQTPKHLITATGQRVTLRCSPRSGDLSVYWYQQSLDQGLQFLIQYYNGEERAKGNILERFSAQQFPDLHSELNLSSLELGDSALYFCASSESRDSGNTIYFGEGSWLTVVEDLNKVFPPEVAVFEPSEAEISHTQKATLVCLATGFFPDHVELSWWVNGKEVHSGVSTDPQPLKEQPALNDSRYCLSSRLRVSATFWQNPRNHFRCQVQFYGLSENDEWTQDRAKPVTQIVSAEAWGRADCGFTSVSYQQGVLSATILYEILLGKATLYAVLVSALVLMAMVKRKDF

SEQ ID NO: 77 - protein, 114 aa, synthetic construct
DSGVTQTPKHLITATGQRVTLRCSPRSGDLSVYWYQQSLDQGLQFLIQYYNGEERAKGNILERFSAQQFPDLHSELNLSSLELGDSALYFCASSESRDSGNTIYFGEGSWLTVV

SEQ ID NO: 78 - protein, 5 aa, synthetic construct
SGDLS

SEQ ID NO: 79 - protein, 6 aa, synthetic construct
YYNGEE

SEQ ID NO: 80 - protein, 13 aa, synthetic construct
ASSESRDSGNTIY

SEQ ID NO: 81 - protein, 273 aa, synthetic construct
METLLGVSLVILWLQLARVNSQQGEEDPQALSIQEGENATMNCSYKTSINNLQWYRQNSGRGLVHLILIRSNEREKHSGRLRVTLDTSKKSSSLLITASRAADTASYFCATDSGGGADGLTFGKGTHLIIQPYIQNPDPAVYQLRDSKSSDKSVCLFTDFDSQTNVSQSKDSDVYITDKTVLDMRSMDFKSNSAVAWSNKSDFACANAFNNSIIPEDTFFPSPESSCDVKLVEKSFETDTNLNFQNLSVIGFRILLLKVAGFNLLMTLRLWSS

SEQ ID NO: 82 - protein, 112 aa, synthetic construct
SQQGEEDPQALSIQEGENATMNCSYKTSINNLQWYRQNSGRGLVHLILIRSNEREKHSGRLRVTLDTSKKSSSLLITASRAADTASYFCATDSGGGADGLTFGKGTHLIIQP

SEQ ID NO: 83 - protein, 5 aa, synthetic construct
TSINN

SEQ ID NO: 84 - protein, 7 aa, synthetic construct
IRSNERE

SEQ ID NO: 85 - protein, 12 aa, synthetic construct
ATDSGGGADGLT

SEQ ID NO: 86 - protein, 310 aa, synthetic construct
MGFRLLCCVAFCLLGAGPVDSGVTQTPKHLITATGQRVTLRCSPRSGDLSVYWYQQSLDQGLQFLIQYYNGEERAKGNILERFSAQQFPDLHSELNLSSLELGDSALYFCASTPGRDSGNTIYFGEGSWLTVVEDLNKVFPPEVAVFEPSEAEISHTQKATLVCLATGFFPDHVELSWWVNGKEVHSGVSTDPQPLKEQPALNDSRYCLSSRLRVSATFWQNPRNHFRCQVQFYGLSENDEWTQDRAKPVTQIVSAEAWGRADCGFTSVSYQQGVLSATILYEILLGKATLYAVLVSALVLMAMVKRKDF

SEQ ID NO: 87 - protein, 114 aa, synthetic construct
DSGVTQTPKHLITATGQRVTLRCSPRSGDLSVYWYQQSLDQGLQFLIQYYNGEERAKGNILERFSAQQFPDLHSELNLSSLELGDSALYFCASTPGRDSGNTIYFGEGSWLTVV

SEQ ID NO: 88 - protein, 5 aa, synthetic construct
SGDLS

SEQ ID NO: 89 - protein, 6 aa, synthetic construct
YYNGEE

SEQ ID NO: 90 - protein, 13 aa, synthetic construct
ASTPGRDSGNTIY

SEQ ID NO: 91 - protein, 9 aa, synthetic construct
VVGAVGVGK

SEQ ID NO: 92 - protein, 10 aa, synthetic construct
VVVGAVGVGK

SEQ ID NO: 93 - protein, 9 aa, synthetic construct
VVGAGGVGK

SEQ ID NO: 94 - protein, 10 aa, synthetic construct
VVVGAGGVGK